European Patent Application EP 4 464 381 A1, published November 20, 2024. Title: MICA ANTIBODY WITH AFFINITY MATURATION AND USE THEREOF. Applicant: Hefei TG ImmunoPharma Co., Ltd. The sequence listing filed with the application follows.

SEQUENCE LISTING (27 sequences)

SEQ ID NO: 1 - protein, 9 aa, synthetic construct
GFSLTTYGG

SEQ ID NO: 2 - protein, 7 aa, synthetic construct
IWTDGWT

SEQ ID NO: 3 - protein, 13 aa, synthetic construct
ARKGHGYYYAMDY

SEQ ID NO: 4 - protein, 7 aa, synthetic construct
SSVSSSY

SEQ ID NO: 5 - protein, 6 aa, synthetic construct
STSNLI

SEQ ID NO: 6 - protein, 9 aa, synthetic construct
HQYHRSPFT

SEQ ID NO: 7 - protein, 119 aa, synthetic construct
QVQLQESGPGLVKPSETLSLTCTVSGFSLTTYGGHWIRQPPGKGLEWIGMIWTDGWTDYNAAFISRVTISVDTSKNQFSLKLSSVTAADTAVYYCARKGHGYYYAMDYWGQGTLVTVSS

SEQ ID NO: 8 - protein, 108 aa, synthetic construct
EIVLTQSPGTLSLSPGERATLSCTASSSVSSSYLHWYQQKPGQAPRLLIYSTSNLISGIPDRFSGSGSGTDFTLTISRLEPEDFAVYYCHQYHRSPFTFGQGTKLEIK

SEQ ID NO: 9 - protein, 119 aa, synthetic construct
QVQLQESGPGLVKPSETLSLTCTVSGFSLTTYGVHWIRQPPGKGLEWIGMIWTDGTTDYNAAFISRVTISVDTSKNQFSLKLSSVTAADTAVYYCARKGHGYYYAMDYWGQGTLVTVSS

SEQ ID NO: 10 - protein, 108 aa, synthetic construct
EIVLTQSPGTLSLSPGERATLSCTASSSVSSSYLHWYQQKPGQAPRLLIYSTSNLASGIPDRFSGSGSGTDFTLTISRLEPEDFAVYYCHQYHRSPFTFGQGTKLEIK

SEQ ID NO: 11 - protein, 449 aa, synthetic construct
QVQLQESGPGLVKPSETLSLTCTVSGFSLTTYGVHWIRQPPGKGLEWIGMIWTDGTTDYNAAFISRVTISVDTSKNQFSLKLSSVTAADTAVYYCARKGHGYYYAMDYWGQGTLVTVSSASTKGPSVFPLAPSSKSTSGGTAALGCLVKDYFPEPVTVSWNSGALTSGVHTFPAVLQSSGLYSLSSVVTVPSSSLGTQTYICNVNHKPSNTKVDKKVEPKSCDKTHTCPPCPAPELLGGPSVFLFPPKPKDTLMISRTPEVTCVVVDVSHEDPEVKFNWYVDGVEVHNAKTKPREEQYNSTYRVVSVLTVLHQDWLNGKEYKCKVSNKALPAPIEKTISKAKGQPREPQVYTLPPSREEMTKNQVSLTCLVKGFYPSDIAVEWESNGQPENNYKTTPPVLDSDGSFFLYSKLTVDKSRWQQGNVFSCSVMHEALHNHYTQKSLSLSPGK

SEQ ID NO: 12 - protein, 215 aa, synthetic construct
EIVLTQSPGTLSLSPGERATLSCTASSSVSSSYLHWYQQKPGQAPRLLIYSTSNLASGIPDRFSGSGSGTDFTLTISRLEPEDFAVYYCHQYHRSPFTFGQGTKLEIKRTVAAPSVFIFPPSDEQLKSGTASVVCLLNNFYPREAKVQWKVDNALQSGNSQESVTEQDSKDSTYSLSSTLTLSKADYEKHKVYACEVTHQGLSSPVTKSFNRGEC

SEQ ID NO: 13 - protein, 449 aa, synthetic construct
QVQLQESGPGLVKPSETLSLTCTVSGFSLTTYGGHWIRQPPGKGLEWIGMIWTDGWTDYNAAFISRVTISVDTSKNQFSLKLSSVTAADTAVYYCARKGHGYYYAMDYWGQGTLVTVSSASTKGPSVFPLAPSSKSTSGGTAALGCLVKDYFPEPVTVSWNSGALTSGVHTFPAVLQSSGLYSLSSVVTVPSSSLGTQTYICNVNHKPSNTKVDKKVEPKSCDKTHTCPPCPAPELLGGPSVFLFPPKPKDTLMISRTPEVTCVVVDVSHEDPEVKFNWYVDGVEVHNAKTKPREEQYNSTYRVVSVLTVLHQDWLNGKEYKCKVSNKALPAPIEKTISKAKGQPREPQVYTLPPSREEMTKNQVSLTCLVKGFYPSDIAVEWESNGQPENNYKTTPPVLDSDGSFFLYSKLTVDKSRWQQGNVFSCSVMHEALHNHYTQKSLSLSPGK

SEQ ID NO: 14 - protein, 215 aa, synthetic construct
EIVLTQSPGTLSLSPGERATLSCTASSSVSSSYLHWYQQKPGQAPRLLIYSTSNLISGIPDRFSGSGSGTDFTLTISRLEPEDFAVYYCHQYHRSPFTFGQGTKLEIKRTVAAPSVFIFPPSDEQLKSGTASVVCLLNNFYPREAKVQWKVDNALQSGNSQESVTEQDSKDSTYSLSSTLTLSKADYEKHKVYACEVTHQGLSSPVTKSFNRGEC

SEQ ID NO: 15 - protein, 449 aa, synthetic construct
QVQLQESGPGLVKPSETLSLTCTVSGFSLTTYGGHWIRQPPGKGLEWIGMIWTDGWTDYNAAFISRVTISVDTSKNQFSLKLSSVTAADTAVYYCARKGHGYYYAMDYWGQGTLVTVSSASTKGPSVFPLAPSSKSTSGGTAALGCLVKDYFPEPVTVSWNSGALTSGVHTFPAVLQSSGLYSLSSVVTVPSSSLGTQTYICNVNHKPSNTKVDKKVEPKSCDKTHTCPPCPAPEAAGGPSVFLFPPKPKDTLMISRTPEVTCVVVDVSHEDPEVKFNWYVDGVEVHNAKTKPREEQYNSTYRVVSVLTVLHQDWLNGKEYKCKVSNKALPAPIEKTISKAKGQPREPQVYTLPPSREEMTKNQVSLTCLVKGFYPSDIAVEWESNGQPENNYKTTPPVLDSDGSFFLYSKLTVDKSRWQQGNVFSCSVMHEALHNHYTQKSLSLSPGK

SEQ ID NO: 16 - protein, 449 aa, synthetic construct
QVQLQESGPGLVKPSETLSLTCTVSGFSLTTYGGHWIRQPPGKGLEWIGMIWTDGWTDYNAAFISRVTISVDTSKNQFSLKLSSVTAADTAVYYCARKGHGYYYAMDYWGQGTLVTVSSASTKGPSVFPLAPSSKSTSGGTAALGCLVKDYFPEPVTVSWNSGALTSGVHTFPAVLQSSGLYSLSSVVTVPSSSLGTQTYICNVNHKPSNTKVDKKVEPKSCDKTHTCPPCPAPELLGGPDVFLFPPKPKDTLMISRTPEVTCVVVDVSHEDPEVKFNWYVDGVEVHNAKTKPREEQYNSTYRVVSVLTVLHQDWLNGKEYKCKVSNKALPLPEEKTISKAKGQPREPQVYTLPPSREEMTKNQVSLTCLVKGFYPSDIAVEWESNGQPENNYKTTPPVLDSDGSFFLYSKLTVDKSRWQQGNVFSCSVMHEALHNHYTQKSLSLSPGK

SEQ ID NO: 17 - protein, 451 aa, synthetic construct
QVQLVESGGGLVKPGGSLRLSCAASGFTFSNYAMSWIRQAPGKGLEWVSYISPGGDYIYYADSVKGRFTISRDNAKNSLYLQMNSLRAEDTAVYYCTTDRRHYGSYAMDYWGQGTLVTVSSASTKGPSVFPLAPSSKSTSGGTAALGCLVKDYFPEPVTVSWNSGALTSGVHTFPAVLQSSGLYSLSSVVTVPSSSLGTQTYICNVNHKPSNTKVDKKVEPKSCDKTHTCPPCPAPELLGGPSVFLFPPKPKDTLMISRTPEVTCVVVDVSHEDPEVKFNWYVDGVEVHNAKTKPREEQYNSTYRVVSVLTVLHQDWLNGKEYKCKVSNKALPAPIEKTISKAKGQPREPQVYTLPPSREEMTKNQVSLTCLVKGFYPSDIAVEWESNGQPENNYKTTPPVLDSDGSFFLYSKLTVDKSRWQQGNVFSCSVMHEALHNHYTQKSLSLSPGK

SEQ ID NO: 18 - protein, 219 aa, synthetic construct
DIVMTQSPLSLPVTPGEPASISCRSSKSLLHSNLNTYLYWFLQKPGQSPQILIYRMSNLASGVPDRFSGSGSGTAFTLKISRVEAEDVGVYYCMQHLEYPFTFGPGTKLEIKRTVAAPSVFIFPPSDEQLKSGTASVVCLLNNFYPREAKVQWKVDNALQSGNSQESVTEQDSKDSTYSLSSTLTLSKADYEKHKVYACEVTHQGLSSPVTKSFNRGEC

SEQ ID NO: 19 - protein, 447 aa, synthetic construct
EIQLVQSGAEVKKPGASVKVSCKASGYAFTSQNIYWVRQAPGQGLEWIGYIEPYNVVPMYNPKFKGRATLTVDKSTSTAYLELSSLRSEDTAVYYCARSGSSNFDYWGQGTLVTVSSASTKGPSVFPLAPSSKSTSGGTAALGCLVKDYFPEPVTVSWNSGALTSGVHTFPAVLQSSGLYSLSSVVTVPSSSLGTQTYICNVNHKPSNTKVDKKVEPKSCDKTHTCPPCPAPELLGGPSVFLFPPKPKDTLMISRTPEVTCVVVDVSHEDPEVKFNWYVDGVEVHNAKTKPREEQYNSTYRVVSVLTVLHQDWLNGKEYKCKVSNKALPAPIEKTISKAKGQPREPQVYTLPPSREEMTKNQVSLTCLVKGFYPSDIAVEWESNGQPENNYKTTPPVLDSDGSFFLYSKLTVDKSRWQQGNVFSCSVMHEALHNHYTQKSLSLSPGK

SEQ ID NO: 20 - protein, 215 aa, synthetic construct
DIQLTQSPSSLSASVGDRVTITCSASSSISSHYLHWYQQKPGKSPKLLIYRTSNLASGVPSRFSGSGSGTDYTLTISSLQPEDFATYYCQQGSSLPLTFGQGTKVEIKRTVAAPSVFIFPPSDEQLKSGTASVVCLLNNFYPREAKVQWKVDNALQSGNSQESVTEQDSKDSTYSLSSTLTLSKADYEKHKVYACEVTHQGLSSPVTKSFNRGEC

SEQ ID NO: 21 - protein, 383 aa, synthetic construct
MGLGPVFLLLAGIFPFAPPGAAAEPHSLRYNLTVLSWDGSVQSGFLTEVHLDGQPFLRCDRQKCRAKPQGQWAEDVLGNKTWDRETRDLTGNGKDLRMTLAHIKDQKEGLHSLQEIRVCEIHEDNSTRSSQHFYYDGELFLSQNLETKEWTMPQSSRAQTLAMNVRNFLKEDAMKTKTHYHAMHADCLQELRRYLKSGVVLRRTVPPMVNVTRSEASEGNITVTCRASGFYPWNITLSWRQDGVSLSHDTQQWGDVLPDGNGTYQTWVATRICQGEEQRFTCYMEHSGNHSTHPVPSGKVLVLQSHWQTFHVSAVAAAAIFVIIIFYVRCCKKKTSAAEGPELVSLQVLDQHPVGTSDHRDATQLGFQPLMSDLGSTGSTEGA

SEQ ID NO: 22 - protein, 336 aa, synthetic construct
RTVPPMVNVTRSEASEGNITVTCRASGFYPWNITLSWRQDGVSLSHDTQQWGDVLPDGNGTYQTWVATRICQGEEQRFTCYMEHSGNHSTHPVPSGKVLVLQSHWPKSCDKTHTCPPCPAPELLGGPSVFLFPPKPKDTLMISRTPEVTCVVVAVSHEDPEVKFNWYVDGVEVHNAKTKPREEQYASTYRVVSVLTVLHQDWLNGKEYKCKVSNKALPAPIEKTISKAKGQPREPQVYTLPPSREEMTKNQVSLTCLVKGFYPSDIAVEWESNGQPENNYKTTPPVLDSDGSFFLYSKLTVDKSRWQQGNVFSCSVMHEALHNHYTQKSLSLSPGK

SEQ ID NO: 23 - protein, 336 aa, synthetic construct
RRVPPMVNVTRSEASEGNITVTCRASSFYPRNITLTWRQDGVSLSHDTQQWGDVLPDGNGTYQTWVATRICQGEEQRFTCYMEHSGNHSTHPVPSGKVLVLQSHWPKSCDKTHTCPPCPAPELLGGPSVFLFPPKPKDTLMISRTPEVTCVVVAVSHEDPEVKFNWYVDGVEVHNAKTKPREEQYASTYRVVSVLTVLHQDWLNGKEYKCKVSNKALPAPIEKTISKAKGQPREPQVYTLPPSREEMTKNQVSLTCLVKGFYPSDIAVEWESNGQPENNYKTTPPVLDSDGSFFLYSKLTVDKSRWQQGNVFSCSVMHEALHNHYTQKSLSLSPGK

SEQ ID NO: 24 - protein, 335 aa, synthetic construct
RTVPPMVNVTCSEVSEGNITVTCRASSFYPRNITLTWRQDGVSLSHNTQQWGDVLPDGNGTYQTWVATRIRQGEEQRFTCYMEHSGNHGTHPVSGKVLVLQSHWPKSCDKTHTCPPCPAPELLGGPSVFLFPPKPKDTLMISRTPEVTCVVVAVSHEDPEVKFNWYVDGVEVHNAKTKPREEQYASTYRVVSVLTVLHQDWLNGKEYKCKVSNKALPAPIEKTISKAKGQPREPQVYTLPPSREEMTKNQVSLTCLVKGFYPSDIAVEWESNGQPENNYKTTPPVLDSDGSFFLYSKLTVDKSRWQQGNVFSCSVMHEALHNHYTQKSLSLSPGK

SEQ ID NO: 25 - protein, 336 aa, synthetic construct
RTVPPMVNVTRSEASEGNITVTCRASSFYPRNIILTWRQDGVSLSHDTQQWGGVLPDGNGTYQTWVATRICRGEEQRFTCYMEHSGNHSTHPVPSGKVLVLQSHWPKSCDKTHTCPPCPAPELLGGPSVFLFPPKPKDTLMISRTPEVTCVVVAVSHEDPEVKFNWYVDGVEVHNAKTKPREEQYASTYRVVSVLTVLHQDWLNGKEYKCKVSNKALPAPIEKTISKAKGQPREPQVYTLPPSREEMTKNQVSLTCLVKGFYPSDIAVEWESNGQPENNYKTTPPVLDSDGSFFLYSKLTVDKSRWQQGNVFSCSVMHEALHNHYTQKSLSLSPGK

SEQ ID NO: 26 - protein, 336 aa, synthetic construct
RTVPPMVNVTCSEVSEGNITVTCRASSFYPRNITLTWRQDGVSLSHNTQQWGDVLPDGNGTYQTWVATRIRQGEEQRFTCYMEHSGNHGTHPVPSGKVLVLQSQRPKSCDKTHTCPPCPAPELLGGPSVFLFPPKPKDTLMISRTPEVTCVVVAVSHEDPEVKFNWYVDGVEVHNAKTKPREEQYASTYRVVSVLTVLHQDWLNGKEYKCKVSNKALPAPIEKTISKAKGQPREPQVYTLPPSREEMTKNQVSLTCLVKGFYPSDIAVEWESNGQPENNYKTTPPVLDSDGSFFLYSKLTVDKSRWQQGNVFSCSVMHEALHNHYTQKSLSLSPGK

SEQ ID NO: 27 - protein, 336 aa, synthetic construct
RTVPPMVNVTCSEVSEGNITVTCRASSFYPRNITLTWRQDGVSLSHNTQQWGDVLPDGNGTYQTWVATRIRQGEEQRFTCYMEHSGNHGTHPVPSGKVLALQSQWPKSCDKTHTCPPCPAPELLGGPSVFLFPPKPKDTLMISRTPEVTCVVVAVSHEDPEVKFNWYVDGVEVHNAKTKPREEQYASTYRVVSVLTVLHQDWLNGKEYKCKVSNKALPAPIEKTISKAKGQPREPQVYTLPPSREEMTKNQVSLTCLVKGFYPSDIAVEWESNGQPENNYKTTPPVLDSDGSFFLYSKLTVDKSRWQQGNVFSCSVMHEALHNHYTQKSLSLSPGK